European Patent Specification EP 3 822 355 B1, published May 20, 2026. Title: ANTI-CANCER COMPOSITION. Applicant: Genemedicine Co.,Ltd. The sequence listing filed with the application follows.

SEQUENCE LISTING (20 sequences)

SEQ ID NO: 1 - DNA, 759 bp, Homo sapiens
atgtggccccctgggtcagcctcccagccaccgccctcacctgccgcggccacaggtctgcatccagcggctcgccctgtgtccctgcagtgccggctcagcatgtgtccagcgcgcagcctcctccttgtggctaccctggtcctcctggaccacctcagtttggccagaaacctccccgtggccactccagacccaggaatgttcccatgccttcaccactcccaaaacctgctgagggccgtcagcaacatgctccagaaggccagacaaactctagaattttacccttgcacttctgaagagattgatcatgtagatatcacaaaagataaaaccagcacagtggaggcctgtttaccattggaattaaccaagaatgagagttgcctaaattccagagagacctctttcataactaatgggagttgcctggcctccagaaagacctcttttatgatggccctgtgccttagtagtatttatgaagacttgaagatgtaccaggtggagttcaagaccatgaatgcaaagcttctgatggatcctaagaggcagatctttctagatcaaaacatgctggcagttattgatgagctgatgcaggccctgaatttcaacagtgagactgtgccacaaaaatcctcccttgaagaaccggatttttataaaactaaaatcaagctctgcatacttcttcatgctttcagaattcgggcagtgactattgatagagtgatgagctatctgaatgcttcc

SEQ ID NO: 2 - DNA, 921 bp, Homo sapiens
atatgggaactgaagaaagatgtttatgtcgtagaattggattggtatccggatgcccctggagaaatggtggtcctcacctgtgacacccctgaagaagatggtatcacctggaccttggaccagagcagtgaggtcttaggctctggcaaaaccctgaccatccgagtcaaagagtttggagatgctggccagtacacctgtcacaaaggaggcgaggttctaagccattcgctcctgctgcttcacaaaaaggaagatggaatttggtccactgatattttaaaggaccagaaagaacccaaaaataagacctttctaagatgcgaggccaagaattattctggacgtttcacctgctggtggctgacgacaatcagtactgatttgacattcagtgtcaaaagcagcagaggctcttctgacccccaaggggtgacgtgcggagctgctacactctctgcagagagagtcagaggggacaacaaggagtatgagtactcagtggagtgccaggaggacagtgcctgcccagctgctgaggagagtctgcccattgaggtcatggtggatgccgttcacaagctcaagtatgaaaactacaccagcagcttcttcatcagggacatcatcaaacctgacccacccaagaacttgcagctgaagccattaaagaattctcggcaggtggaggtcagctgggagtaccctgacacctggagtactccacattcctacttctccctgacattctgcgttcaggtccagggcaagagcaagagagaaaagaaagatagagtcttcacggacaagacctcagccacggtcatctgccgcaaaaatgccagcattagcgtgcgggcccaggaccgctactatagctcatcttggagcgaatgggcatctgtgccctgcagttag

SEQ ID NO: 3 - DNA, 1725 bp, Artificial
  Human IL-12 (p35-linker-p40)
atgtggccccctgggtcagcctcccagccaccgccctcacctgccgcggccacaggtctgcatccagcggctcgccctgtgtccctgcagtgccggctcagcatgtgtccagcgcgcagcctcctccttgtggctaccctggtcctcctggaccacctcagtttggccagaaacctccccgtggccactccagacccaggaatgttcccatgccttcaccactcccaaaacctgctgagggccgtcagcaacatgctccagaaggccagacaaactctagaattttacccttgcacttctgaagagattgatcatgtagatatcacaaaagataaaaccagcacagtggaggcctgtttaccattggaattaaccaagaatgagagttgcctaaattccagagagacctctttcataactaatgggagttgcctggcctccagaaagacctcttttatgatggccctgtgccttagtagtatttatgaagacttgaagatgtaccaggtggagttcaagaccatgaatgcaaagcttctgatggatcctaagaggcagatctttctagatcaaaacatgctggcagttattgatgagctgatgcaggccctgaatttcaacagtgagactgtgccacaaaaatcctcccttgaagaaccggatttttataaaactaaaatcaagctctgcatacttcttcatgctttcagaattcgggcagtgactattgatagagtgatgagctatctgaatgcttccggtggcggtggctcgggcggtggtgggtcgggtggcggcggatctatatgggaactgaagaaagatgtttatgtcgtagaattggattggtatccggatgcccctggagaaatggtggtcctcacctgtgacacccctgaagaagatggtatcacctggaccttggaccagagcagtgaggtcttaggctctggcaaaaccctgaccatccgagtcaaagagtttggagatgctggccagtacacctgtcacaaaggaggcgaggttctaagccattcgctcctgctgcttcacaaaaaggaagatggaatttggtccactgatattttaaaggaccagaaagaacccaaaaataagacctttctaagatgcgaggccaagaattattctggacgtttcacctgctggtggctgacgacaatcagtactgatttgacattcagtgtcaaaagcagcagaggctcttctgacccccaaggggtgacgtgcggagctgctacactctctgcagagagagtcagaggggacaacaaggagtatgagtactcagtggagtgccaggaggacagtgcctgcccagctgctgaggagagtctgcccattgaggtcatggtggatgccgttcacaagctcaagtatgaaaactacaccagcagcttcttcatcagggacatcatcaaacctgacccacccaagaacttgcagctgaagccattaaagaattctcggcaggtggaggtcagctgggagtaccctgacacctggagtactccacattcctacttctccctgacattctgcgttcaggtccagggcaagagcaagagagaaaagaaagatagagtcttcacggacaagacctcagccacggtcatctgccgcaaaaatgccagcattagcgtgcgggcccaggaccgctactatagctcatcttggagcgaatgggcatctgtgccctgcagttag

SEQ ID NO: 4 - DNA, 762 bp, Homo sapiens
atgtggccccctgggtcagcctcccagccaccgccctcacctgccgcggccacaggtctgcatccagcggctcgccctgtgtccctgcagtgccggctcagcatgtgtccagcgcgcagcctcctccttgtggctaccctggtcctcctggaccacctcagtttggccagaaacctccccgtggccactccagacccaggaatgttcccatgccttcaccactcccaaaacctgctgagggccgtcagcaacatgctccagaaggccagacaaactctagaattttacccttgcacttctgaagagattgatcatgaagatatcacaaaagataaaaccagcacagtggaggcctgtttaccattggaattaaccaagaatgagagttgcctaaattccagagagacctctttcataactaatgggagttgcctggcctccagaaagacctcttttatgatggccctgtgccttagtagtatttatgaagacttgaagatgtaccaggtggagttcaagaccatgaatgcaaagcttctgatggatcctaagaggcagatctttctagatcaaaacatgctggcagttattgatgagctgatgcaggccctgaatttcaacagtgagactgtgccacaaaaatcctcccttgaagaaccggatttttataaaactaaaatcaagctctgcatacttcttcatgctttcagaattcgggcagtgactattgatagagtgatgagctatctgaatgcttcctaa

SEQ ID NO: 5 - DNA, 987 bp, Homo sapiens
atgtgtcaccagcagttggtcatctcttggttttccctggtttttctggcatctcccctcgtggccatatgggaactgaagaaagatgtttatgtcgtagaattggattggtatccggatgcccctggagaaatggtggtcctcacctgtgacacccctgaagaagatggtatcacctggaccttggaccagagcagtgaggtcttaggctctggcaaaaccctgaccatccaagtcaaagagtttggagatgctggccagtacacctgtcacaaaggaggcgaggttctaagccattcgctcctgctgcttcacaaaaaggaagatggaatttggtccactgatattttaaaggaccagaaagaacccaaaaataagacctttctaagatgcgaggccaagaattattctggacgtttcacctgctggtggctgacgacaatcagtactgatttgacattcagtgtcaaaagcagcagaggctcttctgacccccaaggggtgacgtgcggagctgctacactctctgcagagagagtcagaggggacaacaaggagtatgagtactcagtggagtgccaggaggacagtgcctgcccagctgctgaggagagtctgcccattgaggtcatggtggatgccgttcacaagctcaagtatgaaaactacaccagcagcttcttcatcagggacatcatcaaacctgacccacccaagaacttgcagctgaagccattaaagaattctcggcaggtggaggtcagctgggagtaccctgacacctggagtactccacattcctacttctccctgacattctgcgttcaggtccagggcaagagcaagagagaaaagaaagatagagtcttcacggacaagacctcagccacggtcatctgccgcaaaaatgccagcattagcgtgcgggcccaggaccgctactatagctcatcttggagcgaatgggcatctgtgccctgcagttag

SEQ ID NO: 6 - DNA, 2331 bp, Artificial
  Human IL-12 (p35-lRES-p40)
atgtggccccctgggtcagcctcccagccaccgccctcacctgccgcggccacaggtctgcatccagcggctcgccctgtgtccctgcagtgccggctcagcatgtgtccagcgcgcagcctcctccttgtggctaccctggtcctcctggaccacctcagtttggccagaaacctccccgtggccactccagacccaggaatgttcccatgccttcaccactcccaaaacctgctgagggccgtcagcaacatgctccagaaggccagacaaactctagaattttacccttgcacttctgaagagattgatcatgaagatatcacaaaagataaaaccagcacagtggaggcctgtttaccattggaattaaccaagaatgagagttgcctaaattccagagagacctctttcataactaatgggagttgcctggcctccagaaagacctcttttatgatggccctgtgccttagtagtatttatgaagacttgaagatgtaccaggtggagttcaagaccatgaatgcaaagcttctgatggatcctaagaggcagatctttctagatcaaaacatgctggcagttattgatgagctgatgcaggccctgaatttcaacagtgagactgtgccacaaaaatcctcccttgaagaaccggatttttataaaactaaaatcaagctctgcatacttcttcatgctttcagaattcgggcagtgactattgatagagtgatgagctatctgaatgcttcctaagcccccccccctaacgttactggccgaagccgcttggaataaggccggtgtgcgtttgtctatatgttattttccaccatattgccgtcttttggcaatgtgagggcccggaaacctggccctgtcttcttgacgagcattcctagctaggggtctttcccctctcgccaaaggaatgcaaggtctgttgaatgtcgtgaaggaagcagttcctctggaagcttcttgaagacaaacaacgtctgtagcgaccctttgcaggcagcggaaccccccacctggcgacaggtgcctctgcggccaaaagccacgtgtataagatacacctgcaaaggcggcacaaccccagtgccacgttgtgagttggatagttgtggaaagagtcaaatggctctcctcaagcgtattcaacaaggggctgaaggatgcccagaaggtaccccattgtatgggatctgatctggggcctcggtgcacatgctttacatgtgtttagtcgaggttaaaaaaacgtctaggccccccgaaccacggggacgtggttttcctttgaaaaacacgatgataatatggccacaaccaatgtgtcaccagcagttggtcatctcttggttttccctggtttttctggcatctcccctcgtggccatatgggaactgaagaaagatgtttatgtcgtagaattggattggtatccggatgcccctggagaaatggtggtcctcacctgtgacacccctgaagaagatggtatcacctggaccttggaccagagcagtgaggtcttaggctctggcaaaaccctgaccatccaagtcaaagagtttggagatgctggccagtacacctgtcacaaaggaggcgaggttctaagccattcgctcctgctgcttcacaaaaaggaagatggaatttggtccactgatattttaaaggaccagaaagaacccaaaaataagacctttctaagatgcgaggccaagaattattctggacgtttcacctgctggtggctgacgacaatcagtactgatttgacattcagtgtcaaaagcagcagaggctcttctgacccccaaggggtgacgtgcggagctgctacactctctgcagagagagtcagaggggacaacaaggagtatgagtactcagtggagtgccaggaggacagtgcctgcccagctgctgaggagagtctgcccattgaggtcatggtggatgccgttcacaagctcaagtatgaaaactacaccagcagcttcttcatcagggacatcatcaaacctgacccacccaagaacttgcagctgaagccattaaagaattctcggcaggtggaggtcagctgggagtaccctgacacctggagtactccacattcctacttctccctgacattctgcgttcaggtccagggcaagagcaagagagaaaagaaagatagagtcttcacggacaagacctcagccacggtcatctgccgcaaaaatgccagcattagcgtgcgggcccaggaccgctactatagctcatcttggagcgaatgggcatctgtgccctgcagttag

SEQ ID NO: 7 - DNA, 645 bp, Mus musculus
atgtgtcaatcacgctacctcctctttttggccacccttgccctcctaaaccacctcagtttggccagggtcattccagtctctggacctgccaggtgtcttagccagtcccgaaacctgctgaagaccacagatgacatggtgaagacggccagagaaaaactgaaacattattcctgcactgctgaagacatcgatcatgaagacatcacacgggaccaaaccagcacattgaagacctgtttaccactggaactacacaagaacgagagttgcctggctactagagagacttcttccacaacaagagggagctgcctgcccccacagaagacgtctttgatgatgaccctgtgccttggtagcatctatgaggacttgaagatgtaccagacagagttccaggccatcaacgcagcacttcagaatcacaaccatcagcagatcattctagacaagggcatgctggtggccatcgatgagctgatgcagtctctgaatcataatggcgagactctgcgccagaaacctcctgtgggagaagcagacccttacagagtgaaaatgaagctctgcatcctgcttcacgccttcagcacccgcgtcgtgaccatcaacagggtgatgggctatctgagctccgcc

SEQ ID NO: 8 - DNA, 1005 bp, Mus musculus
tgtcctcagaagctaaccatctcctggtttgccatcgttttgctggtgtctccactcatggccatgtgggagctggagaaagacgtttatgttgtagaggtggactggactcccgatgcccctggagaaacagtgaacctcacctgtgacacgcctgaagaagatgacatcacctggacctcagaccagagacatggagtcataggctctggaaagaccctgaccatcactgtcaaagagtttctagatgctggccagtacacctgccacaaaggaggcgagactctgagccactcacatctgctgctccacaagaaggaaaatggaatttggtccactgaaattttaaaaaatttcaaaaacaagactttcctgaagtgtgaagcaccaaattactccggacggttcacgtgctcatggctggtgcaaagaaacatggacttgaagttcaacatcaagagcagtagcagttcccctgactctcgggcagtgacatgtggaatggcgtctctgtctgcagagaaggtcacactggaccaaagggactatgagaagtattcagtgtcctgccaggaggatgtcacctgcccaactgccgaggagaccctgcccattgaactggcgttggaagcacggcagcagaataaatatgagaactacagcaccagcttcttcatcagggacatcatcaaaccagacccgcccaagaacttgcagatgaagcctttgaagaactcacaggtggaggtcagctgggagtaccctgactcctggagcactccccattcctacttctccctcaagttctttgttcgaatccagcgcaagaaagaaaagatgaaggagacagaggaggggtgtaaccagaaaggtgcgttcctcgtagagaagacatctaccgaagtccaatgcaaaggcgggaatgtctgcgtgcaagctcaggatcgctattacaattcctcatgcagcaagtgggcatgtgttccctgcagggtccgatcctag

SEQ ID NO: 9 - DNA, 1695 bp, Artificial
  Mouse IL-12 (p35-linker-p40)
atgtgtcaatcacgctacctcctctttttggccacccttgccctcctaaaccacctcagtttggccagggtcattccagtctctggacctgccaggtgtcttagccagtcccgaaacctgctgaagaccacagatgacatggtgaagacggccagagaaaaactgaaacattattcctgcactgctgaagacatcgatcatgaagacatcacacgggaccaaaccagcacattgaagacctgtttaccactggaactacacaagaacgagagttgcctggctactagagagacttcttccacaacaagagggagctgcctgcccccacagaagacgtctttgatgatgaccctgtgccttggtagcatctatgaggacttgaagatgtaccagacagagttccaggccatcaacgcagcacttcagaatcacaaccatcagcagatcattctagacaagggcatgctggtggccatcgatgagctgatgcagtctctgaatcataatggcgagactctgcgccagaaacctcctgtgggagaagcagacccttacagagtgaaaatgaagctctgcatcctgcttcacgccttcagcacccgcgtcgtgaccatcaacagggtgatgggctatctgagctccgccggtggcggtggctcgggcggtggtgggtcgggtggcggcggatcttgtcctcagaagctaaccatctcctggtttgccatcgttttgctggtgtctccactcatggccatgtgggagctggagaaagacgtttatgttgtagaggtggactggactcccgatgcccctggagaaacagtgaacctcacctgtgacacgcctgaagaagatgacatcacctggacctcagaccagagacatggagtcataggctctggaaagaccctgaccatcactgtcaaagagtttctagatgctggccagtacacctgccacaaaggaggcgagactctgagccactcacatctgctgctccacaagaaggaaaatggaatttggtccactgaaattttaaaaaatttcaaaaacaagactttcctgaagtgtgaagcaccaaattactccggacggttcacgtgctcatggctggtgcaaagaaacatggacttgaagttcaacatcaagagcagtagcagttcccctgactctcgggcagtgacatgtggaatggcgtctctgtctgcagagaaggtcacactggaccaaagggactatgagaagtattcagtgtcctgccaggaggatgtcacctgcccaactgccgaggagaccctgcccattgaactggcgttggaagcacggcagcagaataaatatgagaactacagcaccagcttcttcatcagggacatcatcaaaccagacccgcccaagaacttgcagatgaagcctttgaagaactcacaggtggaggtcagctgggagtaccctgactcctggagcactccccattcctacttctccctcaagttctttgttcgaatccagcgcaagaaagaaaagatgaaggagacagaggaggggtgtaaccagaaaggtgcgttcctcgtagagaagacatctaccgaagtccaatgcaaaggcgggaatgtctgcgtgcaagctcaggatcgctattacaattcctcatgcagcaagtgggcatgtgttccctgcagggtccgatcctag

SEQ ID NO: 10 - DNA, 4227 bp, Homo sapiens
atgaaggcccccgctgtgcttgcacctggcatcctcgtgctcctgtttaccttggtgcagaggagcaatggggagtgtaaagaggcactagcaaagtccgagatgaatgtgaatatgaagtatcagcttcccaacttcaccgcggaaacacccatccagaatgtcattctacatgagcatcacattttccttggtgccactaactacatttatgttttaaatgaggaagaccttcagaaggttgctgagtacaagactgggcctgtgctggaacacccagattgtttcccatgtcaggactgcagcagcaaagccaatttatcaggaggtgtttggaaagataacatcaacatggctctagttgtcgacacctactatgatgatcaactcattagctgtggcagcgtcaacagagggacctgccagcgacatgtctttccccacaatcatactgctgacatacagtcggaggttcactgcatattctccccacagatagaagagcccagccagtgtcctgactgtgtggtgagcgccctgggagccaaagtcctttcatctgtaaaggaccggttcatcaacttctttgtaggcaataccataaattcttcttatttcccagatcatccattgcattcgatatcagtgagaaggctaaaggaaacgaaagatggttttatgtttttgacggaccagtcctacattgatgttttacctgagttcagagattcttaccccattaagtatgtccatgcctttgaaagcaacaattttatttacttcttgacggtccaaagggaaactctagatgctcagacttttcacacaagaataatcaggttctgttccataaactctggattgcattcctacatggaaatgcctctggagtgtattctcacagaaaagagaaaaaagagatccacaaagaaggaagtgtttaatatacttcaggctgcgtatgtcagcaagcctggggcccagcttgctagacaaataggagccagcctgaatgatgacattcttttcggggtgttcgcacaaagcaagccagattctgccgaaccaatggatcgatctgccatgtgtgcattccctatcaaatatgtcaacgacttcttcaacaagatcgtcaacaaaaacaatgtgagatgtctccagcatttttacggacccaatcatgagcactgctttaataggacacttctgagaaattcatcaggctgtgaagcgcgccgtgatgaatatcgaacagagtttaccacagctttgcagcgcgttgacttattcatgggtcaattcagcgaagtcctcttaacatctatatccaccttcattaaaggagacctcaccatagctaatcttgggacatcagagggtcgcttcatgcaggttgtggtttctcgatcaggaccatcaacccctcatgtgaattttctcctggactcccatccagtgtctccagaagtgattgtggagcatacattaaaccaaaatggctacacactggttatcactgggaagaagatcacgaagatcccattgaatggcttgggctgcagacatttccagtcctgcagtcaatgcctctctgccccaccctttgttcagtgtggctggtgccacgacaaatgtgtgcgatcggaggaatgcctgagcgggacatggactcaacagatctgtctgcctgcaatctacaaggttttcccaaatagtgcaccccttgaaggagggacaaggctgaccatatgtggctgggactttggatttcggaggaataataaatttgatttaaagaaaactagagttctccttggaaatgagagctgcaccttgactttaagtgagagcacgatgaatacattgaaatgcacagttggtcctgccatgaataagcatttcaatatgtccataattatttcaaatggccacgggacaacacaatacagtacattctcctatgtggatcctgtaataacaagtatttcgccgaaatacggtcctatggctggtggcactttacttactttaactggaaattacctaaacagtgggaattctagacacatttcaattggtggaaaaacatgtactttaaaaagtgtgtcaaacagtattcttgaatgttataccccagcccaaaccatttcaactgagtttgctgttaaattgaaaattgacttagccaaccgagagacaagcatcttcagttaccgtgaagatcccattgtctatgaaattcatccaaccaaatcttttattagtacttggtggaaagaacctctcaacattgtcagttttctattttgctttgccagtggtgggagcacaataacaggtgttgggaaaaacctgaattcagttagtgtcccgagaatggtcataaatgtgcatgaagcaggaaggaactttacagtggcatgtcaacatcgctctaattcagagataatctgttgtaccactccttccctgcaacagctgaatctgcaactccccctgaaaaccaaagcctttttcatgttagatgggatcctttccaaatactttgatctcatttatgtacataatcctgtgtttaagccttttgaaaagccagtgatgatctcaatgggcaatgaaaatgtactggaaattaagggaaatgatattgaccctgaagcagttaaaggtgaagtgttaaaagttggaaataagagctgtgagaatatacacttacattctgaagccgttttatgcacggtccccaatgacctgctgaaattgaacagcgagctaaatatagagtggaagcaagcaatttcttcaaccgtccttggaaaagtaatagttcaaccagatcagaatttcacaggattgattgctggtgttgtctcaatatcaacagcactgttattactacttgggtttttcctgtggctgaaaaagagaaagcaaattaaagatctgggcagtgaattagttcgctacgatgcaagagtacacactcctcatttggataggcttgtaagtgcccgaagtgtaagcccaactacagaaatggtttcaaatgaatctgtagactaccgagctacttttccagaagatcagtttcctaattcatctcagaacggttcatgccgacaagtgcagtatcctctgacagacatgtcccccatcctaactagtggggactctgatatatccagtccattactgcaaaatactgtccacattgacctcagtgctctaaatccagagctggtccaggcagtgcagcatgtagtgattgggcccagtagcctgattgtgcatttcaatgaagtcataggaagagggcattttggttgtgtatatcatgggactttgttggacaatgatggcaagaaaattcactgtgctgtgaaatccttgaacagaatcactgacataggagaagtttcccaatttctgaccgagggaatcatcatgaaagattttagtcatcccaatgtcctctcgctcctgggaatctgcctgcgaagtgaagggtctccgctggtggtcctaccatacatgaaacatggagatcttcgaaatttcattcgaaatgagactcataatccaactgtaaaagatcttattggctttggtcttcaagtagccaaagcgatgaaatatcttgcaagcaaaaagtttgtccacagagacttggctgcaagaaactgtatgctggatgaaaaattcacagtcaaggttgctgattttggtcttgccagagacatgtatgataaagaatactatagtgtacacaacaaaacaggtgcaaagctgccagtgaagtggatggctttggaaagtctgcaaactcaaaagtttaccaccaagtcagatgtgtggtcctttggcgtcgtcctctgggagctgatgacaagaggagccccaccttatcctgacgtaaacacctttgatataactgtttacttgttgcaagggagaagactcctacaacccgaatactgcccagaccccttatatgaagtaatgctaaaatgctggcaccctaaagccgaaatgcgcccatccttttctgaactggtgtcccggatatcagcgatcttctctactttcattggggagcactatgtccatgtgaacgctacttatgtgaacgtaaaatgtgtcgctccgtatccttctctgttgtcatcagaagataacgctgatgatgaggtggacacacgaccagcctccttctgggagacatcatag

SEQ ID NO: 11 - DNA, 6652 bp, Mus musculus
gctcggcggggttcggcccgggccgcaggtgacccggacggcctcgccgcccgcagcgtccgagcccgggtgaccctgtgcggagccagatgctgggcgaccgctgactcgctggagaagggcggagcgcgcgggtggtccccagccggctgacttcggcgccgcgcgctccgggcaccccaaggtacaaactccagccgcgtcgatcaggcacccagcctctcccagcccctctgctttctttgttccactaagggaactggctactgctctggaggacaagaccaccgaggatggctgtggagagaaagctgacggtgtagcagaacgcttggcatgtgatcaactcctcacaatgaaggctcccaccgtgctggcacctggcattctggtgctgctgttgtccttggtgcagaggagccatggggagtgcaaggaggccctagtgaagtctgagatgaacgtgaacatgaagtatcagctccccaacttcacggcagaaacccccatccagaatgtcgtcctacacggccatcatatttatctcggagccacaaactacatttatgttttaaatgacaaagaccttcagaaggtatccgaattcaagaccgggcccgtgttggaacacccagattgtttaccttgtcgggactgcagcagcaaagccaattcatcaggaggggtttggaaagacaacatcaacatggctctgcttgttgacacatactatgatgatcaactcattagctgtggcagtgtcaacagagggacttgccagcggcatgtccttcctcctgacaattctgctgacatccagtctgaggtccactgcatgttctccccagaagaggagtcagggcagtgtcctgactgtgtagtgagtgccctcggagccaaagtcctcctgtcggaaaaggaccggttcatcaatttctttgtggggaatacgatcaattcctcctatcctcctggttattcactgcattcgatatcggtgagacggctgaaggaaacccaagatggttttaagtttttgacagaccagtcctatattgatgtcttaccagaattccaagattcctaccccataaagtacatacatgccttcgaaagcaaccattttatttactttctgactgtccaaaaggaaactctagatgctcagacttttcatacaagaataatcaggttctgttccgtagactctgggttgcactcctacatggaaatgcccctggaatgcatcctgacagaaaaaagaaggaagagatccacaagggaagaagtgtttaatatcctccaagccgcgtatgtcagtaaaccaggggccaatcttgctaagcaaataggagctagcccttctgatgacattctcttcggggtgtttgcacaaagcaagccagattctgctgaacctgtgaatcgatcagcagtctgtgcattccccatcaaatatgtcaatgacttcttcaacaagattgtcaacaaaaacaacgtgagatgtctccagcatttttacggacccaaccatgagcactgtttcaataggaccctgctgagaaactcttccggctgtgaagcgcgcagtgacgagtatcggacagagtttaccacggctttgcagcgcgtcgacttattcatgggccggcttaaccaagtgctcctgacatccatctccaccttcatcaaaggtgacctcaccattgctaatctagggacgtcagaaggtcgcttcatgcaggtggtgctctctcgaacagcacacctcactcctcatgtgaacttcctcctggactcccatcctgtatctccagaagttattgttgagcatccatcaaatcaaaatggctatacattggttgtcacaggaaagaagatcaccaagattccattgaatggcctgggctgtggacatttccaatcctgcagtcagtgcctctctgccccttactttatacagtgtggctggtgccacaatcaatgtgtgcgttttgatgaatgccccagcggtacatggactcaagagatctgtctgccggcggtttataaggtgttccccaccagcgcgccccttgaaggaggaacagtgttgaccatatgtggctgggactttggattcaggaagaataataaatttgatttaaggaaaaccaaagttctgcttggcaacgagagctgtaccttgaccttaagcgagagcacgacaaatacgttgaaatgcacagttggtcccgcgatgagtgagcacttcaatgtgtctgtaattatctcaaacagtcgagagacgacgcaatacagtgcattctcctatgtagatcctgtaataacaagcatttctccgaggtacggccctcaggctggaggcaccttactcactcttactgggaaatacctcaacagtggcaattctagacacatttcaattggagggaaaacatgtactttaaaaagtgtatcagatagtattcttgaatgctacaccccagcccaaactacctctgatgagtttcctgtgaaattgaagattgacttggctaaccgagagaccagcagcttcagttaccgggaagaccccgttgtctatgaaatccacccgaccaaatcttttattagtggtggaagcacaataacgggtattgggaagaccctgaactcggttagcctcccaaagctggtaatagatgtgcatgaagtgggtgtgaactacacagtggcatgtcagcatcgctcaaattcagagatcatctgctgcactactccttcactgaaacagctgggcctgcaactccccctgaagaccaaagccttcttcctgttagacgggattctttccaaacactttgatctcacttatgtgcataatcctgtgtttgagccttttgaaaagccagtaatgatctcaataggcaatgaaaatgtagtggaaattaagggaaacaatattgaccctgaagcagttaaaggtgaagtgttaaaagttggaaatcagagctgcgagagtctccactggcactctggagctgtgttgtgtacagtccccagtgacctgctcaaactgaacagcgagctaaatatagagtggaagcaagcagtctcttcaactgttcttggaaaagtgatcgttcaaccggatcagaattttgcaggattgatcattggtgcggtctcaatatcagtagtagttttgttattatccgggctcttcctgtggatgagaaagagaaagcataaagatctgggcagtgaattagttcgctatgacgcaagagtacacactcctcatttggataggcttgtaagtgcccgaagtgtaagtccaactacagagatggtttcaaatgagtctgtagactacagagctacttttccagaagaccagtttcccaactcctctcagaatggagcatgcagacaagtgcaataccctctgacagacctgtcccctatcctgacaagtggagactctgatatatccagcccattactacaaaatactgttcacattgacctcagtgctctaaatccagagctggtccaagcagttcagcacgtagtgattggacccagcagcctgattgtgcatttcaatgaagtcataggaagagggcattttggctgtgtctatcatgggactttgctggacaatgacggaaagaaaattcactgtgctgtgaaatccttaaatagaatcacagatatagaagaggtctcccagtttctgactgagggaatcatcatgaaagacttcagccatcccaatgttctctcactcttgggaatctgcctgaggagtgaagggtctcctctggtggtcctgccctatatgaagcatggagatctgcgaaatttcattcgaaacgagactcataatccaactgtgaaagatcttataggatttggccttcaagtagccaaaggcatgaaatatcttgccagcaaaaagtttgtccacagagacttagctgcaagaaactgcatgttggatgaaaaattcactgtcaaggttgctgatttcggtcttgccagagacatgtacgataaagagtactatagtgtccacaacaagacgggtgccaagctaccagtaaagtggatggctttagagagtctgcaaacgcagaagttcaccaccaagtcagatgtgtggtcctttggtgtgctcctctgggagctcatgacgagaggagcccctccttatcccgacgtgaacacatttgatatcactatctacctgttgcaaggcagaagactcttgcaaccagaatactgtccagacgccttgtacgaagtgatgctaaaatgctggcaccccaaagcggaaatgcgcccgtccttttccgaactggtctccaggatatcctcaatcttctccacgttcattggggaacactacgtccacgtgaacgctacttatgtgaatgtaaaatgtgttgctccatatccttctctgttgccatcccaagacaacattgatggcgaggggaacacatgatgaatgagaggtccaccagcccacttccaagaaacagttctggcccaaaccagactatcccttccccaacagttctcactgcctggcctttggaaggtcacttaacatttgttgttgttttgttttgttttttgttttgcttttgcggtaactgcaccactatgaaacattgacttgctatttcaaattcctggattctaaggaatttctcatctgacaatggaacagaaatagaagcatggcccccacaggctggggaccagtggcaacctgcagctacaacactcctatctcagcggaattctaaatctcagttctggcttaaaagttttaaaaataagatatatatacatatatatatccaatacaatgaactttgaagatttctcagaaaactcagaagaaacgccctctttcaggataaatgtggtgttcctagcaggctgcttgttgaaattccagtgttttaaaaatatttttgttgtgttgcagtcgtgaacattttccatttctgatgttgtctgcccatcaggcaaacattcccttttaaatgcttatatacacattccttaggttggaagaatatccacggacaatgcacttatttttaaacgagcatgacatgaggtgtgtttataaattatcagggattttatgtattgtacatagatgacaataggaaattgtttatttcaagaaatagctttgttacagtaaaatatttgtcatttaaaacccagctgtttagcaaggagtgttggctcacacctacaatcccagcatttgggaagctgaggcaagcagattaccacaagtttgaaaccaaccttggctgcatacagatgatgtatatataggccagcatgggttacactgtctgtcttagcaaacaaaatttcaactgtttgagaaagattttgttctgatctaatgaatgtggacatttaaattttttatctgttttttaatggcaactttggaaataagtaacttgcggtgataaatctttttaaaggcaactcagtattttttaaaggacaaaataaactgactgaagggttcgctacttccagtcacaacctgtgtatagaagaaagaaagggtcagtgatcgagaatcagacactctcgttcaggaggaggcttctcgcctgaaacaattgcacccaacacttttggggaagtctcatttttgcattaggacatattttaggttaaacaaaagcatattttagaaacagacaaaagccaactgaaaatcgtggatgaatagttactctggacaggacttttgacatgtcttgctctgtggaattttgtgcttactactgtatagtgcatgtggcttaggttaccctagctggttttgtccgtgtaaacattgaaagtattatatttttatagaaatgtttatttttaatgatgtaagaaaaattttccttaggccgcagaaatcctgcactgtgagcatttcagaagaggtatgtgagacccagttcaacgacagcatgattttttaaatggctgtaagttatgataaggaaatgtactgattgccagtgcactccaccctcattacgtcaccaggacttgaagccaagggttaagagggcaagctatgacatgggtgtgtggtctgctgaaacccaatcgttgaacttggctgttgttacaggaaaatgatggcatcaacaggtctttgatggtggtggagcatatcagaacacataaggaactgtagcccagatttatttcaattcaaatattactgcttcgtaattatgaagagtagtgcaaatttacagagcactgtcaaagactgacagaaaaaaaaaagatctgctctgtagaaagaattgtctgccattacagggtcaagaaaatgaatgcgccaataacagtaagagctgtggaagacacccatacctgtatatacatgctcgagaaagctgtaatgtgaaaatcatgttctctatttatgactcttcctagggcaatgtgtctggacagattgtaagagtaagtcattttcctaaagaattagatatttgtcactgcctatacctgcagttgagctgaatggtactccatgtgttaataattgttctgatgaatcatacagttgaaataaagtgacgtaacatcttgtatactgtga

SEQ ID NO: 12 - DNA, 62 bp, Artificial
  shRNA SEQ. for Human c-met
caaactagagttctccttggaattcaagagattccaaggagaactctagtttttttttggaa

SEQ ID NO: 13 - DNA, 21 bp, Artificial
  Target sequence in Human c-met
aaactagagttctccttggaa

SEQ ID NO: 14 - DNA, 69 bp, Artificial
  shRNA SEQ for Mouse c-met
ctccacgtgaacgctacttatgtgaattcaagagattcacataagtagcgttcacgtggatttttggaa

SEQ ID NO: 15 - DNA, 25 bp, Artificial
  Target sequence in Mouse c-met
tccacgtgaacgctacttatgtgaa

SEQ ID NO: 16 - DNA, 63 bp, Artificial
  CRISPR gRNA SEQ for Human c-met
aatttctactaagtgtagataatttctactaagtgtagatcactccccattgctcctctgcac

SEQ ID NO: 17 - DNA, 23 bp, Artificial
  Target sequence in Human c-met
gtgcagaggagcaatggggagtg

SEQ ID NO: 18 - DNA, 3684 bp, Artificial
  Lbcpf1 SEQ
atgagcaagctggagaagtttacaaactgctactccctgtctaagaccctgaggttcaaggccatccctgtgggcaagacccaggagaacatcgacaataagcggctgctggtggaggacgagaagagagccgaggattataagggcgtgaagaagctgctggatcgctactatctgtcttttatcaacgacgtgctgcacagcatcaagctgaagaatctgaacaattacatcagcctgttccggaagaaaaccagaaccgagaaggagaataaggagctggagaacctggagatcaatctgcggaaggagatcgccaaggccttcaagggcaacgagggctacaagtccctgtttaagaaggatatcatcgagacaatcctgccagagttcctggacgataaggacgagatcgccctggtgaacagcttcaatggctttaccacagccttcaccggcttctttgataacagagagaatatgttttccgaggaggccaagagcacatccatcgccttcaggtgtatcaacgagaatctgacccgctacatctctaatatggacatcttcgagaaggtggacgccatctttgataagcacgaggtgcaggagatcaaggagaagatcctgaacagcgactatgatgtggaggatttctttgagggcgagttctttaactttgtgctgacacaggagggcatcgacgtgtataacgccatcatcggcggcttcgtgaccgagagcggcgagaagatcaagggcctgaacgagtacatcaacctgtataatcagaaaaccaagcagaagctgcctaagtttaagccactgtataagcaggtgctgagcgatcgggagtctctgagcttctacggcgagggctatacatccgatgaggaggtgctggaggtgtttagaaacaccctgaacaagaacagcgagatcttcagctccatcaagaagctggagaagctgttcaagaattttgacgagtactctagcgccggcatctttgtgaagaacggccccgccatcagcacaatctccaaggatatcttcggcgagtggaacgtgatccgggacaagtggaatgccgagtatgacgatatccacctgaagaagaaggccgtggtgaccgagaagtacgaggacgatcggagaaagtccttcaagaagatcggctccttttctctggagcagctgcaggagtacgccgacgccgatctgtctgtggtggagaagctgaaggagatcatcatccagaaggtggatgagatctacaaggtgtatggctcctctgagaagctgttcgacgccgattttgtgctggagaagagcctgaagaagaacgacgccgtggtggccatcatgaaggacctgctggattctgtgaagagcttcgagaattacatcaaggccttctttggcgagggcaaggagacaaacagggacgagtccttctatggcgattttgtgctggcctacgacatcctgctgaaggtggaccacatctacgatgccatccgcaattatgtgacccagaagccctactctaaggataagttcaagctgtattttcagaaccctcagttcatgggcggctgggacaaggataaggagacagactatcgggccaccatcctgagatacggctccaagtactatctggccatcatggataagaagtacgccaagtgcctgcagaagatcgacaaggacgatgtgaacggcaattacgagaagatcaactataagctgctgcccggccctaataagatgctgccaaaggtgttcttttctaagaagtggatggcctactataaccccagcgaggacatccagaagatctacaagaatggcacattcaagaagggcgatatgtttaacctgaatgactgtcacaagctgatcgacttctttaaggatagcatctcccggtatccaaagtggtccaatgcctacgatttcaacttttctgagacagagaagtataaggacatcgccggcttttacagagaggtggaggagcagggctataaggtgagcttcgagtctgccagcaagaaggaggtggataagctggtggaggagggcaagctgtatatgttccagatctataacaaggacttttccgataagtctcacggcacacccaatctgcacaccatgtacttcaagctgctgtttgacgagaacaatcacggacagatcaggctgagcggaggagcagagctgttcatgaggcgcgcctccctgaagaaggaggagctggtggtgcacccagccaactcccctatcgccaacaagaatccagataatcccaagaaaaccacaaccctgtcctacgacgtgtataaggataagaggttttctgaggaccagtacgagctgcacatcccaatcgccatcaataagtgccccaagaacatcttcaagatcaatacagaggtgcgcgtgctgctgaagcacgacgataacccctatgtgatcggcatcgataggggcgagcgcaatctgctgtatatcgtggtggtggacggcaagggcaacatcgtggagcagtattccctgaacgagatcatcaacaacttcaacggcatcaggatcaagacagattaccactctctgctggacaagaaggagaaggagaggttcgaggcccgccagaactggacctccatcgagaatatcaaggagctgaaggccggctatatctctcaggtggtgcacaagatctgcgagctggtggagaagtacgatgccgtgatcgccctggaggacctgaactctggctttaagaatagccgcgtgaaggtggagaagcaggtgtatcagaagttcgagaagatgctgatcgataagctgaactacatggtggacaagaagtctaatccttgtgcaacaggcggcgccctgaagggctatcagatcaccaataagttcgagagctttaagtccatgtctacccagaacggcttcatcttttacatccctgcctggctgacatccaagatcgatccatctaccggctttgtgaacctgctgaaaaccaagtataccagcatcgccgattccaagaagttcatcagctcctttgacaggatcatgtacgtgcccgaggaggatctgttcgagtttgccctggactataagaacttctctcgcacagacgccgattacatcaagaagtggaagctgtactcctacggcaaccggatcagaatcttccggaatcctaagaagaacaacgtgttcgactgggaggaggtgtgcctgaccagcgcctataaggagctgttcaacaagtacggcatcaattatcagcagggcgatatcagagccctgctgtgcgagcagtccgacaaggccttctactctagctttatggccctgatgagcctgatgctgcagatgcggaacagcatcacaggccgcaccgacgtggattttctgatcagccctgtgaagaactccgacggcatcttctacgatagccggaactatgaggcccaggagaatgccatcctgccaaagaacgccgacgccaatggcgcctataacatcgccagaaaggtgctgtgggccatcggccagttcaagaaggccgaggacgagaagctggataaggtgaagatcgccatctctaacaaggagtggctggagtacgcccagaccagcgtgaagcac

SEQ ID NO: 19 - DNA, 45 bp, Artificial
  linker sequence for IL-12
ggtggcggtggctcgggcggtggtgggtcgggtggcggcggatct

SEQ ID NO: 20 - DNA, 582 bp, Artificial
  lRES sequence
gcccccccccctaacgttactggccgaagccgcttggaataaggccggtgtgcgtttgtctatatgttattttccaccatattgccgtcttttggcaatgtgagggcccggaaacctggccctgtcttcttgacgagcattcctagctaggggtctttcccctctcgccaaaggaatgcaaggtctgttgaatgtcgtgaaggaagcagttcctctggaagcttcttgaagacaaacaacgtctgtagcgaccctttgcaggcagcggaaccccccacctggcgacaggtgcctctgcggccaaaagccacgtgtataagatacacctgcaaaggcggcacaaccccagtgccacgttgtgagttggatagttgtggaaagagtcaaatggctctcctcaagcgtattcaacaaggggctgaaggatgcccagaaggtaccccattgtatgggatctgatctggggcctcggtgcacatgctttacatgtgtttagtcgaggttaaaaaaacgtctaggccccccgaaccacggggacgtggttttcctttgaaaaacacgatgataatatggccacaacca